European Patent Application EP 4 644 570 A1, published November 5, 2025. Title: 一种解旋酶突变体及其制备方法和在高通量测序中的应用. Applicant: 深圳华大生命科学研究院. The sequence listing filed with the application follows.

SEQUENCE LISTING (8 sequences)

SEQ ID NO: 1 - protein, 454 aa, synthetic construct
MKHDLSSATEEQRYIFTDFIKQAQLALKGDSDYEVFAIQGFAGSGKTWLSALIIDELLELGMKVAVTSPTHKAVRVSLNMLKNNGIDTNSPLMYPGTIHHFLNLKLDHGFADDGTADNVTTKAKLVVNKFNECLEYVDVLIVDEASMVSGELYDHALKTLGDRCKIILFIGDSYQLLPVDDEDSSIFLKDDIFHYKLTKVVRQAEDNIIIAKSQELIKAMDQKTYYPSVNDYFVNITEDTEGIKLLKSNVELFELYFSDFKDKMTGAYTNKVVNQFNEYIRYTLYQETKFICDKDELVFQETYTDSKGNIIVSNGEIIEVATCKLTTDIDKFKIWKIVSKKNELGECVRFNVLDPSSYNEFNDLLDKYLADAKIAKGYDRSKAWKKYFKLKEKYAKVRYNFSSTIHKLQGSTYQNMYFDMRGLDYFYRMNRDNVLRLVYVGITRASDQVFILQD

SEQ ID NO: 2 - DNA, 68 bp, synthetic construct
  source 1..68: mol_type = other DNA
  misc_binding 40..41: bound_moiety = connected by four iSp18 modifications
ttttttttttttttttttttttttttttttttttttttttggttgtttctgttggtgctgatattgct

SEQ ID NO: 3 - DNA, 45 bp, synthetic construct
  source 1..45: mol_type = other DNA
gcaatatcagcaccaacagaaacaacctttgaggcgagcggtcaa

SEQ ID NO: 4 - DNA, 15 bp, synthetic construct
  source 1..15: mol_type = other DNA
  misc_feature 1: note = a cholesterol modification at 5' terminus
ttgaccgctcgcctc

SEQ ID NO: 5 - DNA, 1365 bp, synthetic construct
  source 1..1365: mol_type = other DNA
atgaaacatgatctgagcagcgcaaccgaagaacagcgttatatttttaccgatttcatcaagcaggcccagctggcactgaaaggtgatagcgattatgaagtttttgccatccagggttttgccggtagcggtaaaacctggctgagcgcactgattattgatgaactgctggaactgggtatgaaagttgcagttaccagcccgacccataaagcagttcgtgttagcctgaatatgctgaaaaataacggcattgacaccaacagcccgctgatgtatccgggtaccattcatcattttctgaatctgaaactggaccacggttttgccgatgatggtaccgcagataatgttaccaccaaagcaaaactggttgtgaacaagttcaacgagtgtctggaatacgttgacgttctgatcgttgatgaagcaagcatggttagcggtgaactgtatgatcatgcactgaaaaccctgggtgatcgttgtaaaattattctgtttatcggcgacagctaccagctgctgccggttgatgatgaagatagcagcatttttctgaaggacgacatttttcactacaagctgaccaaagtggtgcgccaggcagaagataatattattattgccaaaagccaggagctgatcaaggcaatggatcagaaaacctattacccgagcgttaatgactatttcgttaacatcaccgaggacaccgaaggcattaaactgctgaaaagcaatgttgagctgttcgaactgtactttagcgacttcaaggataagatgaccggcgcatataccaataaagttgtgaatcagtttaacgagtacatccgctataccctgtatcaggaaaccaaatttatttgcgataaggacgagctggtgttccaggaaacctataccgatagcaaaggtaatattattgtgagcaatggcgagatcatcgaggttgcaacctgtaaactgaccaccgatattgataaattcaagatctggaagatcgtgagcaagaagaacgaactgggtgaatgtgtgcgtttcaatgttctggatccgagcagctataatgaatttaatgatctgctggacaagtacctggccgatgcaaaaattgcaaaaggttatgaccgtagcaaagcctggaaaaaatatttcaagctgaaagagaagtacgccaaggtgcgttacaacttcagcagcaccatccacaagctgcagggtagcacctatcagaatatgtattttgacatgcgcggcctggactatttttatcgcatgaatcgtgataacgtgctgcgcctggtttatgtgggtattacccgtgcaagcgatcaggtttttattctgcaggattaa

SEQ ID NO: 6 - protein, 454 aa, synthetic construct
MKHDLSSATEEQRYIFTDFIKQAQLALKGDSDYEVFAIQGFAGSGKTWLSALIIDELLELGMKVAVTSPTHKAVRVSLNMLKNNGIDTNSPLMYPGTIHHFLNLKLDHGFADDGTADNVTTKAKLVVNKFNEALEYVDVLIVDEASMVSGELYDHALKTLGDRAKIILFIGDSYQLLPVDDEDSSIFLKDDIFHYKLTKVVRQAEDNIIIAKSQELIKAMDQKTYYPSVNDYFVNITEDTEGIKLLKSNVELFELYFSDFKDKMTGAYTNKVVNQFNEYIRYTLYQETKFIADKDELVFQETYTDSKGNIIVSNGEIIEVATAKLTTDIDKFKIWKIVSKKNELGEAVRFNVLDPSSYNEFNDLLDKYLADAKIAKGYDRSKAWKKYFKLKEKYAKVRYNFSSTIHKLQGSTYQNMYFDMRGLDYFYRMNRDNVLRLVYVGITRASDQVFILQD

SEQ ID NO: 7 - protein, 454 aa, synthetic construct
MKHDLSSATEEQRYIFTDFIKQAQLALKGDSDYEVFAIQGFAGSGKTWLSALIIDELLELGMKVAVTSPTHKAVRVSLNMLKNNGIDTNSPLMYPGTIHHFLNLKLDHGFADDGTACNVTTKAKLVVNKFNEALEYVDVLIVDEASMVSGELYDHALKTLGDRAKIILFIGDSYQLLPVDDEDSSIFLKDDIFHYKLTKVVRQAEDNIIIAKSQELIKAMDQKTYYPSVNDYFVNITEDTEGIKLLKSNVELFELYFSDFKDKMTGAYTNKVVNQFNEYIRYTLYQETKFIADKDELVFQETYTDSKGNIIVSNGEIIEVATAKLTTDIDKFKIWKIVSKKNELGEAVRFNVLDPSSYNEFNDLLDKYCADAKIAKGYDRSKAWKKYFKLKEKYAKVRYNFSSTIHKLQGSTYQNMYFDMRGLDYFYRMNRDNVLRLVYVGITRASDQVFILQD

SEQ ID NO: 8 - DNA, 1365 bp, synthetic construct
  source 1..1365: mol_type = other DNA
atgaaacatgatctgagcagcgcgaccgaagaacagcgctatatttttaccgattttatcaagcaggcgcagctggcgctgaaaggcgatagcgattatgaagtgtttgcgattcagggctttgcgggcagcggcaaaacctggttaagcgcgttaattattgatgagctgctggaactgggcatgaaagtggccgtgaccagcccgacccataaagcggttcgtgtgagcctgaacatgctgaaaaacaacggcattgataccaacagcccgctgatgtatccgggcaccattcatcattttctgaacctgaaactggatcatggctttgcggatgatggcaccgcggataacgttaccaccaaagcgaaactggtggtgaacaaatttaacgaagcgctggaatatgtggatgtgctgattgtggatgaagcgagcatggtgagcggcgaactgtatgatcatgcgctgaaaaccctgggcgatcgcgcgaaaattattctgtttattggcgatagctatcagctgctgccggtggatgatgaagatagcagcatttttctgaaagacgacatcttccattacaagctgaccaaggtggtgcgccaggcggaagataacattattattgcgaaaagccaggagctgattaaagcgatggatcagaaaacctattatccgagcgtgaacgattattttgtgaacattaccgaagacaccgaaggcattaaactgctgaaaagcaacgtggaactgtttgaactgtattttagcgattttaaggacaagatgaccggcgcgtataccaacaaagtggtgaaccagtttaacgaatatatccgctataccctgtatcaggaaaccaaatttattgcggataaagacgaactggtgtttcaggaaacctataccgatagcaaaggcaacattattgtgagcaacggcgaaattattgaggtggcgaccgcgaaactgaccaccgatattgataaatttaaaatctggaagatcgtgagcaagaagaacgaactgggcgaagcggtgcgctttaacgtgctggatccgagcagctataacgaatttaacgatctgctggataaatacctggcggatgcgaaaattgcgaaaggctatgatcgcagcaaagcgtggaagaaatattttaaactgaaggagaagtacgcgaaagtgcgctataactttagcagcaccattcataaactgcagggcagcacctatcagaacatgtattttgatatgcgcggcctggattatttttatcgcatgaaccgcgataacgtgctgcgcctggtgtatgtgggcattacccgcgcgagcgatcaggtgtttattctgcaggattaa